European Patent Specification EP 3 822 362 B1, published May 15, 2024. Title: ON-SLIDE STAINING BY PRIMER EXTENSION. Applicant: The Board of Trustees of the Leland Stanford Junior University Samusik, Nikolay Nolan, Garry P Goltsev, Yury. The sequence listing filed with the application follows.

SEQUENCE LISTING (174 sequences)

SEQ ID NO: 1 - DNA, 13 bp, Artificial Sequence
  Synthetic oligonucleotide
  misc_feature (1)..(1): n is uridine
  misc_feature (5)..(5): n is uridine
  misc_feature (9)..(9): n is uridine
  misc_feature (13)..(13): n is uridine
naaanaaanaaan

SEQ ID NO: 2 - DNA, 13 bp, Artificial Sequence
  Synthetic oligonucleotide
atttatttattta

SEQ ID NO: 3 - DNA, 11 bp, Artificial Sequence
  Synthetic oligonucleotide
  misc_feature (1)..(1): n is uridine
  misc_feature (5)..(5): n is uridine
  misc_feature (11)..(11): n is uridine
naacnaacaan

SEQ ID NO: 4 - DNA, 13 bp, Artificial Sequence
  Synthetic oligonucleotide
attgttattgtta

SEQ ID NO: 5 - DNA, 42 bp, Artificial Sequence
  Synthetic oligonucleotide
  misc_feature (42)..(42): c is dideoxycytidine
ttctagggggggggggggtcgtcaagatgctaccgttcaggc

SEQ ID NO: 6 - DNA, 34 bp, Artificial Sequence
  Synthetic oligonucleotide
  misc_feature (1)..(1): linked to an antibody at the 5' end
atagcgctaccctgaacggtagcatcttgacgac

SEQ ID NO: 7 - DNA, 42 bp, Artificial Sequence
  Synthetic oligonucleotide
  misc_feature (42)..(42): c is dideoxycytidine
ttctaacgatctagtcggtcgtcaagatgctaccgttcaggc

SEQ ID NO: 8 - DNA, 35 bp, Artificial Sequence
  Synthetic oligonucleotide
  misc_feature (1)..(1): linked to an antibody at the 5' end
atagcgctacgcctgaacggtagcatcttgacgac

SEQ ID NO: 9 - DNA, 41 bp, Artificial Sequence
  Synthetic oligonucleotide
ttctactctctctctctgtcgtcaagatgctaccgttcagg

SEQ ID NO: 10 - DNA, 35 bp, Artificial Sequence; identical to SEQ ID NO: 8
  Synthetic oligonucleotide
  misc_feature (1)..(1): linked to an antibody at the 5' end

SEQ ID NO: 11 - DNA, 41 bp, Artificial Sequence
  Synthetic oligonucleotide
ttctactcctttcctctgtcgtcaagatgctaccgttcagg

SEQ ID NO: 12 - DNA, 35 bp, Artificial Sequence; identical to SEQ ID NO: 8
  Synthetic oligonucleotide
  misc_feature (1)..(1): linked to an antibody at the 5' end

SEQ ID NO: 13 - DNA, 35 bp, Artificial Sequence; identical to SEQ ID NO: 8
  Synthetic oligonucleotide
  misc_feature (1)..(1): linked to an antibody at the 5' end
  misc_feature (35)..(5): c is dideoxycytidine

SEQ ID NO: 14 - DNA, 52 bp, Artificial Sequence
  Synthetic oligonucleotide
  misc_feature (7)..(27): n is a, c, g, or t
  misc_feature (52)..(52): c is dideoxycytidine
tttttannnnnnnnnnnnnnnnnnnnngtcgtcaagatgctaccgttcaggc

SEQ ID NO: 15 - DNA, 35 bp, Artificial Sequence; identical to SEQ ID NO: 8
  Synthetic oligonucleotide
  misc_feature (1)..(1): linked to an antibody at the 5' end
  misc_feature (35)..(35): c is dideoxycytidine

SEQ ID NO: 16 - DNA, 53 bp, Artificial Sequence
  Synthetic oligonucleotide
  misc_feature (8)..(28): n is a, c, g, or t
  misc_feature (53)..(53): c is dideoxycytidine
tttttacnnnnnnnnnnnnnnnnnnnnngtcgtcaagatgctaccgttcaggc

SEQ ID NO: 17 - DNA, 35 bp, Artificial Sequence; identical to SEQ ID NO: 8
  Synthetic oligonucleotide
  misc_feature (1)..(1): linked to an antibody at the 5' end
  misc_feature (35)..(35): c is dideoxycytidine

SEQ ID NO: 18 - DNA, 54 bp, Artificial Sequence
  Synthetic oligonucleotide
  misc_feature (9)..(29): n is a, c, g, or t
  misc_feature (54)..(54): c is dideoxycytidine
tttttactnnnnnnnnnnnnnnnnnnnnngtcgtcaagatgctaccgttcaggc

SEQ ID NO: 19 - DNA, 35 bp, Artificial Sequence; identical to SEQ ID NO: 8
  Synthetic oligonucleotide
  misc_feature (1)..(1): linked to an antibody at the 5' end
  misc_feature (35)..(5): c is dideoxycytidine

SEQ ID NO: 20 - DNA, 52 bp, Artificial Sequence; identical to SEQ ID NO: 14
  Synthetic oligonucleotide
  misc_feature (7)..(27): n is a, c, g, or t
  misc_feature (52)..(52): c is dideoxycytidine

SEQ ID NO: 21 - DNA, 35 bp, Artificial Sequence; identical to SEQ ID NO: 8
  Synthetic oligonucleotide
  misc_feature (1)..(1): linked to an antibody at the 5' end
  misc_feature (35)..(35): c is dideoxycytidine

SEQ ID NO: 22 - DNA, 53 bp, Artificial Sequence; identical to SEQ ID NO: 16
  Synthetic oligonucleotide
  misc_feature (8)..(28): n is a, c, g, or t
  misc_feature (53)..(53): c is dideoxycytidine

SEQ ID NO: 23 - DNA, 35 bp, Artificial Sequence; identical to SEQ ID NO: 8
  Synthetic oligonucleotide
  misc_feature (1)..(1): linked to an antibody at the 5' end
  misc_feature (35)..(35): c is dideoxycytidine

SEQ ID NO: 24 - DNA, 54 bp, Artificial Sequence; identical to SEQ ID NO: 18
  Synthetic oligonucleotide
  misc_feature (9)..(29): n is a, c, g, or t
  misc_feature (54)..(54): c is dideoxycytidine

SEQ ID NO: 25 - DNA, 35 bp, Artificial Sequence; identical to SEQ ID NO: 8
  Synthetic oligonucleotide
  misc_feature (1)..(1): linked to an antibody at the 5' end
  misc_feature (35)..(35): c is dideoxycytidine

SEQ ID NO: 26 - DNA, 52 bp, Artificial Sequence; identical to SEQ ID NO: 14
  Synthetic oligonucleotide
  misc_feature (7)..(27): n is a, c, g, or t
  misc_feature (52)..(52): c is dideoxycytidine

SEQ ID NO: 27 - DNA, 35 bp, Artificial Sequence; identical to SEQ ID NO: 8
  Synthetic oligonucleotide
  misc_feature (1)..(1): linked to an antibody at the 5' end
  misc_feature (35)..(35): c is dideoxycytidine

SEQ ID NO: 28 - DNA, 53 bp, Artificial Sequence; identical to SEQ ID NO: 16
  Synthetic oligonucleotide
  misc_feature (8)..(28): n is a, c, g, or t
  misc_feature (53)..(53): c is dideoxycytidine

SEQ ID NO: 29 - DNA, 35 bp, Artificial Sequence; identical to SEQ ID NO: 8
  Synthetic oligonucleotide
  misc_feature (1)..(1): linked to an antibody at the 5' end
  misc_feature (35)..(35): c is dideoxycytidine

SEQ ID NO: 30 - DNA, 54 bp, Artificial Sequence; identical to SEQ ID NO: 18
  Synthetic oligonucleotide
  misc_feature (9)..(29): n is a, c, g, or t
  misc_feature (54)..(54): c is dideoxycytidine

SEQ ID NO: 31 - DNA, 24 bp, Artificial Sequence
  Synthetic oligonucleotide
cctgaacggtagcatcttgacgac

SEQ ID NO: 32 - DNA, 19 bp, Artificial Sequence
  Synthetic oligonucleotide
  misc_feature (1)..(1): linked to a quncher at the 5' end
  misc_feature (19)..(19): linked to a fluorophore at the 3' end
aaaaaaaaacgcggcccgg

SEQ ID NO: 33 - DNA, 44 bp, Artificial Sequence
  Synthetic oligonucleotide
ccgggccgcgtttttttttagtcgtcaagatgctaccgttcagg

SEQ ID NO: 34 - DNA, 44 bp, Artificial Sequence
  Synthetic oligonucleotide
  misc_feature (44)..(44): linked to a fluorophore at the 3' end
cctgaacggtagcatcttgacgactaaaaaaaaacgcggcccgg

SEQ ID NO: 35 - DNA, 44 bp, Artificial Sequence; identical to SEQ ID NO: 33
  Synthetic oligonucleotide

SEQ ID NO: 36 - DNA, 24 bp, Artificial Sequence
  Synthetic oligonucleotide
cctgaacggtagcatcttgacgac

SEQ ID NO: 37 - DNA, 19 bp, Artificial Sequence
  Synthetic oligonucleotide
  misc_feature (1)..(1): linked to a quencher at the 5' end
  misc_feature (19)..(19): linked to a fluorophore at the 3' end
aaaaaaaaacgcggcccgg

SEQ ID NO: 38 - DNA, 44 bp, Artificial Sequence; identical to SEQ ID NO: 33
  Synthetic oligonucleotide

SEQ ID NO: 39 - DNA, 24 bp, Artificial Sequence
  Synthetic oligonucleotide
cctgaacggtagcatcttgacgac

SEQ ID NO: 40 - DNA, 19 bp, Artificial Sequence
  Synthetic oligonucleotide
  misc_feature (1)..(1): linked to a quencher at the 5' end
  misc_feature (19)..(19): linked to a fluorophore at the 3' end
aaaaaaaaacgcggcccgg

SEQ ID NO: 41 - DNA, 45 bp, Artificial Sequence
  Synthetic oligonucleotide
ccgggccgcgtttttttttacgtcgtcaagatgctaccgttcagg

SEQ ID NO: 42 - DNA, 24 bp, Artificial Sequence
  Synthetic oligonucleotide
cctgaacggtagcatcttgacgac

SEQ ID NO: 43 - DNA, 19 bp, Artificial Sequence
  Synthetic oligonucleotide
  misc_feature (1)..(1): linked to a quencher at the 5' end
  misc_feature (19)..(19): linked to a fluorophore at the 3' end
aaaaaaaaacgcggcccgg

SEQ ID NO: 44 - DNA, 46 bp, Artificial Sequence
  Synthetic oligonucleotide
ccgggccgcgtttttttttcaggtcgtcaagatgctaccgttcagg

SEQ ID NO: 45 - DNA, 44 bp, Artificial Sequence; identical to SEQ ID NO: 34
  Synthetic oligonucleotide
  misc_feature (44)..(44): linked to a fluorophore at the 3' end

SEQ ID NO: 46 - DNA, 44 bp, Artificial Sequence; identical to SEQ ID NO: 33
  Synthetic oligonucleotide

SEQ ID NO: 47 - DNA, 24 bp, Artificial Sequence
  Synthetic oligonucleotide
cctgaacggtagcatcttgacgac

SEQ ID NO: 48 - DNA, 19 bp, Artificial Sequence
  Synthetic oligonucleotide
  misc_feature (1)..(1): linked to a quencher at the 5' end
  misc_feature (19)..(19): linked to a fluorophore at the 3' end
aaaaaaaaacgcggcccgg

SEQ ID NO: 49 - DNA, 45 bp, Artificial Sequence; identical to SEQ ID NO: 41
  Synthetic oligonucleotide

SEQ ID NO: 50 - DNA, 24 bp, Artificial Sequence
  Synthetic oligonucleotide
cctgaacggtagcatcttgacgac

SEQ ID NO: 51 - DNA, 19 bp, Artificial Sequence
  Synthetic oligonucleotide
  misc_feature (1)..(1): linked to a quencher at the 5' end
  misc_feature (19)..(19): linked to a fluorophore at the 3' end
aaaaaaaaacgcggcccgg

SEQ ID NO: 52 - DNA, 46 bp, Artificial Sequence; identical to SEQ ID NO: 44
  Synthetic oligonucleotide

SEQ ID NO: 53 - DNA, 44 bp, Artificial Sequence; identical to SEQ ID NO: 34
  Synthetic oligonucleotide

SEQ ID NO: 54 - DNA, 44 bp, Artificial Sequence; identical to SEQ ID NO: 33
  Synthetic oligonucleotide

SEQ ID NO: 55 - DNA, 25 bp, Artificial Sequence
  Synthetic oligonucleotide
cctgaacggtagcatcttgacgacg

SEQ ID NO: 56 - DNA, 19 bp, Artificial Sequence
  Synthetic oligonucleotide
  misc_feature (19)..(19): linked to a fluorophore at the 3' end
aaaaaaaaacgcggcccgg

SEQ ID NO: 57 - DNA, 45 bp, Artificial Sequence; identical to SEQ ID NO: 41
  Synthetic oligonucleotide

SEQ ID NO: 58 - DNA, 25 bp, Artificial Sequence
  Synthetic oligonucleotide
cctgaacggtagcatcttgacgacc

SEQ ID NO: 59 - DNA, 19 bp, Artificial Sequence
  Synthetic oligonucleotide
  misc_feature (1)..(1): linked to a quencher at the 5' end
  misc_feature (19)..(19): linked to a fluorophore at the 3' end
aaaaaaaaacgcggcccgg

SEQ ID NO: 60 - DNA, 46 bp, Artificial Sequence; identical to SEQ ID NO: 44
  Synthetic oligonucleotide

SEQ ID NO: 61 - DNA, 44 bp, Artificial Sequence; identical to SEQ ID NO: 34
  Synthetic oligonucleotide

SEQ ID NO: 62 - DNA, 44 bp, Artificial Sequence; identical to SEQ ID NO: 33
  Synthetic oligonucleotide

SEQ ID NO: 63 - DNA, 45 bp, Artificial Sequence
  Synthetic oligonucleotide
  misc_feature (63)..(63): linked to a fluorophore at the 3' end
cctgaacggtagcatcttgacgacgtaaaaaaaaacgcggcccgg

SEQ ID NO: 64 - DNA, 45 bp, Artificial Sequence; identical to SEQ ID NO: 41
  Synthetic oligonucleotide

SEQ ID NO: 65 - DNA, 26 bp, Artificial Sequence
  Synthetic oligonucleotide
cctgaacggtagcatcttgacgacct

SEQ ID NO: 66 - DNA, 19 bp, Artificial Sequence
  Synthetic oligonucleotide
  misc_feature (1)..(1): linked to a quencher at the 5' end
  misc_feature (19)..(19): linked to a fluorophore at the 3' end
aaaaaaaaacgcggcccgg

SEQ ID NO: 67 - DNA, 46 bp, Artificial Sequence; identical to SEQ ID NO: 44
  Synthetic oligonucleotide

SEQ ID NO: 68 - DNA, 34 bp, Artificial Sequence
  Synthetic oligonucleotide
  misc_feature (34)..(34): linked to an antibody at the 3' end
atagagcgagccagtgctagggtgagtggccaag

SEQ ID NO: 69 - DNA, 34 bp, Artificial Sequence; identical to SEQ ID NO: 68
  Synthetic oligonucleotide
  misc_feature (34)..(34): linked to an antibody at the 3' end

SEQ ID NO: 70 - DNA, 16 bp, Artificial Sequence
  Synthetic oligonucleotide
gcactggctcgctcta

SEQ ID NO: 71 - DNA, 34 bp, Artificial Sequence; identical to SEQ ID NO: 68
  Synthetic oligonucleotide
  misc_feature (34)..(34): linked to an antibody at the 3' end

SEQ ID NO: 72 - DNA, 17 bp, Artificial Sequence
  Synthetic oligonucleotide
  misc_feature (17)..(17): linked to Cy5 at the 3' end
gcactggctcgctctan

SEQ ID NO: 73 - DNA, 34 bp, Artificial Sequence; identical to SEQ ID NO: 68
  Synthetic oligonucleotide
  misc_feature (34)..(34): linked to an antibody at the 3' end

SEQ ID NO: 74 - DNA, 8 bp, Artificial Sequence
  Synthetic oligonucleotide
gcactggc

SEQ ID NO: 75 - DNA, 35 bp, Artificial Sequence
  Synthetic oligonucleotide
  misc_feature (35)..(35): linked to an antibody at the 3' end
catagagcgagccagtgctagggtgagtggccaag

SEQ ID NO: 76 - DNA, 17 bp, Artificial Sequence
  Synthetic oligonucleotide
  misc_feature (17)..(17): linked to Cy5 at the 3' end
gcactggctcgctctan

SEQ ID NO: 77 - DNA, 35 bp, Artificial Sequence
  Synthetic oligonucleotide
  misc_feature (35)..(35): linked to an antibody at the 3' end
caatgtccaggccagtgctagggtgagtggccaag

SEQ ID NO: 78 - DNA, 16 bp, Artificial Sequence
  Synthetic oligonucleotide
gcactggctcgctcta

SEQ ID NO: 79 - DNA, 35 bp, Artificial Sequence
  Synthetic oligonucleotide
  misc_feature (35)..(35): linked to an antibody at the 3' end
caagtcagtgaccagtgctagggtgagtggccaag

SEQ ID NO: 80 - DNA, 16 bp, Artificial Sequence
  Synthetic oligonucleotide
gcactggctcgctcta

SEQ ID NO: 81 - DNA, 35 bp, Artificial Sequence
  Synthetic oligonucleotide
  misc_feature (1)..(1): linked to Cy5 at the 5' end
  misc_feature (18)..(35): n is a, c, g, or t
acgtacgctcgtgccgcnnnnnnnnnnnnnnnnnn

SEQ ID NO: 82 - DNA, 17 bp, Artificial Sequence
  Synthetic oligonucleotide
  misc_feature (17)..(17): linked to Cy3 at the 3' end
gcggcacgagcgtacgn

SEQ ID NO: 83 - DNA, 35 bp, Artificial Sequence
  Synthetic oligonucleotide
  misc_feature (1)..(1): linked to Cy5 at the 5' end
  misc_feature (18)..(35): n is a, c, g, or t
acctgcgctcgtgccgcnnnnnnnnnnnnnnnnnn

SEQ ID NO: 84 - DNA, 16 bp, Artificial Sequence
  Synthetic oligonucleotide
gcggcacgagcgtacg

SEQ ID NO: 85 - DNA, 35 bp, Artificial Sequence
  Synthetic oligonucleotide
  misc_feature (1)..(1): linked to Cy5 at the 5' end
  misc_feature (18)..(35): n is a, c, g, or t
agcatcgctcgtgccgcnnnnnnnnnnnnnnnnnn

SEQ ID NO: 86 - DNA, 16 bp, Artificial Sequence
  Synthetic oligonucleotide
gcggcacgagcgtacg

SEQ ID NO: 87 - DNA, 50 bp, Artificial Sequence
  Synthetic oligonucleotide
  misc_feature (1)..(1): linked to an antibody at the 5' end
gaaccggtgagtgggatagcgctacgcctgaacggtagcatcttgacgac

SEQ ID NO: 88 - DNA, 31 bp, Artificial Sequence
  Synthetic oligonucleotide
  misc_feature (31)..(31): c is dideoxycytidine
tttttagtcgtcaagatgctaccgttcaggc

SEQ ID NO: 89 - DNA, 24 bp, Artificial Sequence
  Synthetic oligonucleotide
cctgaacggtagcatcttgacgac

SEQ ID NO: 90 - DNA, 31 bp, Artificial Sequence; identical to SEQ ID NO: 88
  Synthetic oligonucleotide
  misc_feature (31)..(31): c is dideoxycytidine

SEQ ID NO: 91 - DNA, 24 bp, Artificial Sequence
  Synthetic oligonucleotide
cctgaacggtagcatcttgacgac

SEQ ID NO: 92 - DNA, 32 bp, Artificial Sequence
  Synthetic oligonucleotide
  misc_feature (32)..(32): c is dideoxycytidine
tttttatgtcgtcaagatgctaccgttcaggc

SEQ ID NO: 93 - DNA, 24 bp, Artificial sequence
  Synthetic oligonucleotide
cctgaacggtagcatcttgacgac

SEQ ID NO: 94 - DNA, 26 bp, Artificial sequence
  Synthetic oligonucleotide
atgcacgtcgtcaagatgctaccgtt

SEQ ID NO: 95 - DNA, 24 bp, Artificial sequence
  Synthetic oligonucleotide
cctgaacggtagcatcttgacgac

SEQ ID NO: 96 - DNA, 27 bp, Artificial sequence
  Synthetic oligonucleotide
atgcatcgtcgtcaagatgctaccgtt

SEQ ID NO: 97 - DNA, 25 bp, Artificial sequence
  Synthetic oligonucleotide
cctgaacggtagcatcttgacgacg

SEQ ID NO: 98 - DNA, 26 bp, Artificial sequence
  Synthetic oligonucleotide
atgcacgtcgtcaagatgctaccgtt

SEQ ID NO: 99 - DNA, 25 bp, Artificial sequence
  Synthetic oligonucleotide
cctgaacggtagcatcttgacgacg

SEQ ID NO: 100 - DNA, 27 bp, Artificial sequence
  Synthetic oligonucleotide
atgcatcgtcgtcaagatgctaccgtt

SEQ ID NO: 101 - DNA, 30 bp, Artificial sequence
  Synthetic oligonucleotide
cctgaacggtagcatcttgacgacgtgcat

SEQ ID NO: 102 - DNA, 26 bp, Artificial sequence
  Synthetic oligonucleotide
atgcacgtcgtcaagatgctaccgtt

SEQ ID NO: 103 - DNA, 30 bp, Artificial sequence; identical to SEQ ID NO: 101
  Synthetic oligonucleotide

SEQ ID NO: 104 - DNA, 27 bp, Artificial sequence
  Synthetic oligonucleotide
atgcatcgtcgtcaagatgctaccgtt

SEQ ID NO: 105 - DNA, 30 bp, Artificial sequence; identical to SEQ ID NO: 101
  Synthetic oligonucleotide

SEQ ID NO: 106 - DNA, 26 bp, Artificial sequence
  Synthetic oligonucleotide
atgcacgtcgtcaagatgctaccgtt

SEQ ID NO: 107 - DNA, 25 bp, Artificial sequence
  Synthetic oligonucleotide
cctgaacggtagcatcttgacgacg

SEQ ID NO: 108 - DNA, 27 bp, Artificial sequence
  Synthetic oligonucleotide
atgcatcgtcgtcaagatgctaccgtt

SEQ ID NO: 109 - DNA, 29 bp, Artificial sequence
  Synthetic oligonucleotide
cctgaacggtagcatcttgacgactgcat

SEQ ID NO: 110 - DNA, 26 bp, Artificial sequence
  Synthetic oligonucleotide
atgcacgtcgtcaagatgctaccgtt

SEQ ID NO: 111 - DNA, 25 bp, Artificial sequence
  Synthetic oligonucleotide
cctgaacggtagcatcttgacgacg

SEQ ID NO: 112 - DNA, 27 bp, Artificial sequence
  Synthetic oligonucleotide
atgcatcgtcgtcaagatgctaccgtt

SEQ ID NO: 113 - DNA, 30 bp, Artificial sequence; identical to SEQ ID NO: 101
  Synthetic oligonucleotide

SEQ ID NO: 114 - DNA, 26 bp, Artificial sequence
  Synthetic oligonucleotide
atgcacgtcgtcaagatgctaccgtt

SEQ ID NO: 115 - DNA, 26 bp, Artificial sequence
  Synthetic oligonucleotide
cctgaacggtagcatcttgacgacga

SEQ ID NO: 116 - DNA, 27 bp, Artificial sequence
  Synthetic oligonucleotide
atgcatcgtcgtcaagatgctaccgtt

SEQ ID NO: 117 - DNA, 30 bp, Artificial sequence; identical to SEQ ID NO: 101
  Synthetic oligonucleotide

SEQ ID NO: 118 - DNA, 26 bp, Artificial sequence
  Synthetic oligonucleotide
atgcacgtcgtcaagatgctaccgtt

SEQ ID NO: 119 - DNA, 31 bp, Artificial sequence
  Synthetic oligonucleotide
cctgaacggtagcatcttgacgacgatgcat

SEQ ID NO: 120 - DNA, 27 bp, Artificial sequence
  Synthetic oligonucleotide
atgcatcgtcgtcaagatgctaccgtt

SEQ ID NO: 121 - DNA, 30 bp, Artificial sequence; identical to SEQ ID NO: 101
  Synthetic oligonucleotide

SEQ ID NO: 122 - DNA, 26 bp, Artificial sequence
  Synthetic oligonucleotide
atgcacgtcgtcaagatgctaccgtt

SEQ ID NO: 123 - DNA, 31 bp, Artificial sequence; identical to SEQ ID NO: 119
  Synthetic oligonucleotide

SEQ ID NO: 124 - DNA, 27 bp, Artificial sequence
  Synthetic oligonucleotide
atgcatcgtcgtcaagatgctaccgtt

SEQ ID NO: 125 - DNA, 55 bp, Artificial sequence
  Synthetic oligonucleotide
atgctaccgttaattattactgaaacatacactaaagataacattattctgcaag

SEQ ID NO: 126 - DNA, 18 bp, Artificial sequence
  Synthetic oligonucleotide
tgaaacatacactaaaga

SEQ ID NO: 127 - DNA, 13 bp, Artificial sequence
  Synthetic oligonucleotide
gcatcttgcagaa

SEQ ID NO: 128 - DNA, 28 bp, Artificial sequence
  Synthetic oligonucleotide
ttttgttctgcaagatgctaccgttcgg

SEQ ID NO: 129 - DNA, 29 bp, Artificial sequence
  Synthetic oligonucleotide
ttttgtttctgcaagatgctaccgttcgg

SEQ ID NO: 130 - DNA, 30 bp, Artificial sequence
  Synthetic oligonucleotide
ttttgctttctgcaagatgctaccgttcgg

SEQ ID NO: 131 - DNA, 31 bp, Artificial sequence
  Synthetic oligonucleotide
ttttgtctttctgcaagatgctaccgttcgg

SEQ ID NO: 132 - DNA, 33 bp, Artificial sequence
  Synthetic oligonucleotide
ttttgcctctttctgcaagatgctaccgttcgg

SEQ ID NO: 133 - DNA, 36 bp, Artificial sequence
  Synthetic oligonucleotide
ttttgtttcctctttctgcaagatgctaccgttcgg

SEQ ID NO: 134 - DNA, 38 bp, Artificial sequence
  Synthetic oligonucleotide
ttttgcctttcctctttctgcaagatgctaccgttcgg

SEQ ID NO: 135 - DNA, 40 bp, Artificial sequence
  Synthetic oligonucleotide
ttttgttcctttcctctttctgcaagatgctaccgttcgg

SEQ ID NO: 136 - DNA, 41 bp, Artificial sequence
  Synthetic oligonucleotide
ttttgcttcctttcctctttctgcaagatgctaccgttcgg

SEQ ID NO: 137 - DNA, 42 bp, Artificial sequence
  Synthetic oligonucleotide
ttttgtcttcctttcctctttctgcaagatgctaccgttcgg

SEQ ID NO: 138 - DNA, 44 bp, Artificial sequence
  Synthetic oligonucleotide
ttttgcctcttcctttcctctttctgcaagatgctaccgttcgg

SEQ ID NO: 139 - DNA, 28 bp, Artificial sequence
  Synthetic oligonucleotide
ttttattctgcaagatgctaccgttcgg

SEQ ID NO: 140 - DNA, 29 bp, Artificial sequence
  Synthetic oligonucleotide
ttttatttctgcaagatgctaccgttcgg

SEQ ID NO: 141 - DNA, 30 bp, Artificial sequence
  Synthetic oligonucleotide
ttttactttctgcaagatgctaccgttcgg

SEQ ID NO: 142 - DNA, 31 bp, Artificial sequence
  Synthetic oligonucleotide
ttttatctttctgcaagatgctaccgttcgg

SEQ ID NO: 143 - DNA, 33 bp, Artificial sequence
  Synthetic oligonucleotide
ttttacctctttctgcaagatgctaccgttcgg

SEQ ID NO: 144 - DNA, 36 bp, Artificial sequence
  Synthetic oligonucleotide
ttttatttcctctttctgcaagatgctaccgttcgg

SEQ ID NO: 145 - DNA, 38 bp, Artificial sequence
  Synthetic oligonucleotide
ttttacctttcctctttctgcaagatgctaccgttcgg

SEQ ID NO: 146 - DNA, 40 bp, Artificial sequence
  Synthetic oligonucleotide
ttttattcctttcctctttctgcaagatgctaccgttcgg

SEQ ID NO: 147 - DNA, 41 bp, Artificial sequence
  Synthetic oligonucleotide
ttttacttcctttcctctttctgcaagatgctaccgttcgg

SEQ ID NO: 148 - DNA, 42 bp, Artificial sequence
  Synthetic oligonucleotide
ttttatcttcctttcctctttctgcaagatgctaccgttcgg

SEQ ID NO: 149 - DNA, 44 bp, Artificial sequence
  Synthetic oligonucleotide
ttttacctcttcctttcctctttctgcaagatgctaccgttcgg

SEQ ID NO: 150 - DNA, 29 bp, Artificial sequence
  Synthetic oligonucleotide
  misc_feature (29)..(29): n = dideoxyC
ttttattctgcaagatgctaccgttcggn

SEQ ID NO: 151 - DNA, 30 bp, Artificial sequence
  Synthetic oligonucleotide
  misc_feature (30)..(30): n = dideoxyC
ttttatttctgcaagatgctaccgttcggn

SEQ ID NO: 152 - DNA, 31 bp, Artificial sequence
  Synthetic oligonucleotide
  misc_feature (31)..(31): n = dideoxyC
ttttactttctgcaagatgctaccgttcggn

SEQ ID NO: 153 - DNA, 36 bp, Artificial sequence
  Synthetic oligonucleotide
  misc_feature (36)..(36): n = dideoxyC
atagcagtccagccgaacggtagcatcttgcagaan

SEQ ID NO: 154 - DNA, 45 bp, Artificial sequence
  Synthetic oligonucleotide
  misc_feature (45)..(45): n = dideoxyC
ttttagcgattaagcgtgaacttctgcaagatgctaccgttcggn

SEQ ID NO: 155 - DNA, 46 bp, Artificial sequence
  Synthetic oligonucleotide
  misc_feature (46)..(46): n = dideoxyC
ttttatgcgattaagcgtgaacttctgcaagatgctaccgttcggn

SEQ ID NO: 156 - DNA, 47 bp, Artificial sequence
  Synthetic oligonucleotide
  misc_feature (47)..(47): n = dideoxyC
ttttactgcgattaagcgtgaacttctgcaagatgctaccgttcggn

SEQ ID NO: 157 - DNA, 36 bp, Artificial sequence; identical to SEQ ID NO: 153
  Synthetic oligonucleotide
  misc_feature (36)..(36): n = dideoxyC

SEQ ID NO: 158 - DNA, 45 bp, Artificial sequence
  Synthetic oligonucleotide
  misc_feature (45)..(45): n = dideoxyC
ttttacgctaattcgcacttgttctgcaagatgctaccgttcggn

SEQ ID NO: 159 - DNA, 46 bp, Artificial sequence
  Synthetic oligonucleotide
  misc_feature (46)..(46): n = dideoxyC
ttttatcgctaattcgcacttgttctgcaagatgctaccgttcggn

SEQ ID NO: 160 - DNA, 47 bp, Artificial sequence
  Synthetic oligonucleotide
  misc_feature (47)..(47): n = dideoxyC
ttttactcgctaattcgcacttgttctgcaagatgctaccgttcggn

SEQ ID NO: 161 - DNA, 16 bp, Artificial sequence
  Synthetic oligonucleotide
gttcacgcttaatcgc

SEQ ID NO: 162 - DNA, 16 bp, Artificial sequence
  Synthetic oligonucleotide
cgctaattcgcacttg

SEQ ID NO: 163 - DNA, 55 bp, Artificial sequence
  Synthetic oligonucleotide
acattaaaatcctagcacagggactcaattattactgaaacatacactaaagata

SEQ ID NO: 164 - DNA, 34 bp, Artificial sequence
  Synthetic oligonucleotide
ctcatcagcacagctatgatgataatgttatctt

SEQ ID NO: 165 - DNA, 55 bp, Artificial sequence
  Synthetic oligonucleotide
acattatagaactcggcctggatgataattattactgaaacatacactaaagata

SEQ ID NO: 166 - DNA, 32 bp, Artificial sequence
  Synthetic oligonucleotide
ctgattggtcaggattcagataatgttatctt

SEQ ID NO: 167 - DNA, 55 bp, Artificial sequence
  Synthetic oligonucleotide
acattatcaaagctggcaaatcgtccaattattactgaaacatacactaaagata

SEQ ID NO: 168 - DNA, 32 bp, Artificial sequence
  Synthetic oligonucleotide
tggccaatgcaccttgagcctaatgttatctt

SEQ ID NO: 169 - DNA, 55 bp, Artificial sequence
  Synthetic oligonucleotide
acattatgatttccaggttggctttgaattattactgaaacatacactaaagata

SEQ ID NO: 170 - DNA, 32 bp, Artificial sequence
  Synthetic oligonucleotide
atagttggagcgctttgtcataatgttatctt

SEQ ID NO: 171 - DNA, 55 bp, Artificial sequence
  Synthetic oligonucleotide
acattatttcgaagccacgtgacattaattattactgaaacatacactaaagata

SEQ ID NO: 172 - DNA, 32 bp, Artificial sequence
  Synthetic oligonucleotide
ctgtggtgacaggttttccataatgttatctt

SEQ ID NO: 173 - DNA, 19 bp, Artificial sequence
  Synthetic oligonucleotide
catacactaaagataacat

SEQ ID NO: 174 - DNA, 35 bp, Artificial sequence
  Synthetic oligonucleotide
atagcagtccagccgaacggtagcatcttgcagaa